European Patent Application EP 4 733 761 A1, published April 29, 2026. Title: 神経変性疾患に関連するタンパク質および神経変性疾患の治療薬または予防薬のスクリーニング方法. Applicant: 国立研究開発法人産業技術総合研究所. Application JP. The sequence listing filed with the application follows.

SEQUENCE LISTING (7 sequences)

SEQ ID NO: 1 - protein, 40 aa, synthetic construct
  REGION 1..40: note = Dnc-PR20
  MOD_RES 1: note = dansyl-modified
PRPRPRPRPRPRPRPRPRPRPRPRPRPRPRPRPRPRPRPR

SEQ ID NO: 2 - protein, 40 aa, synthetic construct
  REGION 1..40: note = Dnc-GP20
  MOD_RES 1: note = dansyl-modified
GPGPGPGPGPGPGPGPGPGPGPGPGPGPGPGPGPGPGPGP

SEQ ID NO: 3 - protein, 20 aa, synthetic construct
  REGION 1..20: note = Dnc-GA10
  MOD_RES 1: note = dansyl-modified
GAGAGAGAGAGAGAGAGAGA

SEQ ID NO: 4 - protein, 20 aa, synthetic construct
  REGION 1..20: note = Dnc-GR10
  MOD_RES 1: note = dansyl-modified
GRGRGRGRGRGRGRGRGRGR

SEQ ID NO: 5 - protein, 20 aa, synthetic construct
  REGION 1..20: note = Dnc-PR10
  MOD_RES 1: note = dansyl-modified
PRPRPRPRPRPRPRPRPRPR

SEQ ID NO: 6 - protein, 20 aa, synthetic construct
  REGION 1..20: note = Dnc-GP10
  MOD_RES 1: note = dansyl-modified
GPGPGPGPGPGPGPGPGPGP

SEQ ID NO: 7 - protein, 20 aa, synthetic construct
  REGION 1..20: note = Dnc-PA10
  MOD_RES 1: note = dansyl-modified
PAPAPAPAPAPAPAPAPAPA